European Patent Specification EP 3 810 279 B1, published September 13, 2023. Title: Combination Therapy Using a Peptide. Applicant: Cytovation AS. The sequence listing filed with the application follows.

SEQUENCE LISTING (3 sequences)

SEQ ID NO: 1 - protein, 27 aa, Artificial Sequence
  CyPep-1 peptide sequence
YGRKKRRQRRRGKTLRVAKAIYKRYIE

SEQ ID NO: 2 - protein, 15 aa, Homo sapiens
KTLRVAKAIYKRYIE

SEQ ID NO: 3 - protein, 12 aa, Human immunodeficiency virus
YGRKKRRQRRRG